European Patent Application EP 4 742 249 A1, published May 13, 2026. Title: Method of selecting Neoantigen for Development of Personalized Cancer Vaccine. Applicant: LG CHEM, LTD. The sequence listing filed with the application follows.

SEQUENCE LISTING (134 sequences)

SEQ ID NO: 1 - protein, 181 aa, synthetic construct
  REGION 1..181: note = HLA-A0201
SHSMRYFFTSVSRPGRGEPRFIAVGYVDDTQFVRFDSDAASQRMEPRAPWIEQEGPEYWDGETRKVKAHSQTHRVDLGTLRGYYNQSEAGSHTVQRMYGCDVGSDWRFLRGYHQYAYDGKDYIALKEDLRSWTAADMAAQTTKHKWEAAHVAEQLRAYLEGTCVEWLRRYLENGKETLQRT

SEQ ID NO: 2 - protein, 181 aa, synthetic construct
  REGION 1..181: note = HLA-A1101
SHSMRYFYTSVSRPGRGEPRFIAVGYVDDTQFVRFDSDAASQRMEPRAPWIEQEGPEYWDQETRNVKAQSQTDRVDLGTLRGYYNQSEDGSHTIQIMYGCDVGPDGRFLRGYRQDAYDGKDYIALNEDLRSWTAADMAAQITKRKWEAAHAAEQQRAYLEGRCVEWLRRYLENGKETLQRT

SEQ ID NO: 3 - protein, 181 aa, synthetic construct
  REGION 1..181: note = HLA-A2402
SHSMRYFSTSVSRPGRGEPRFIAVGYVDDTQFVRFDSDAASQRMEPRAPWIEQEGPEYWDEETGKVKAHSQTDRENLRIALRYYNQSEAGSHTLQMMFGCDVGSDGRFLRGYHQYAYDGKDYIALKEDLRSWTAADMAAQITKRKWEAAHVAEQQRAYLEGTCVDGLRRYLENGKETLQRT

SEQ ID NO: 4 - protein, 9 aa, synthetic construct
  REGION 1..9: note = neoantigen candidate (A0201) (Melanoma)
YLFNFVVNV

SEQ ID NO: 5 - protein, 9 aa, synthetic construct
  REGION 1..9: note = neoantigen candidate (A0201) (Melanoma)
RLAEFIIGM

SEQ ID NO: 6 - protein, 10 aa, synthetic construct
  REGION 1..10: note = neoantigen candidate (A0201) (Melanoma)
YLFNFVVNVG

SEQ ID NO: 7 - protein, 10 aa, synthetic construct
  REGION 1..10: note = neoantigen candidate (A0201) (Melanoma)
RLAEFIIGMM

SEQ ID NO: 8 - protein, 10 aa, synthetic construct
  REGION 1..10: note = neoantigen candidate (A0201) (Melanoma)
LLTDIIPDGV

SEQ ID NO: 9 - protein, 9 aa, synthetic construct
  REGION 1..9: note = neoantigen candidate (A0201) (Melanoma)
FLALCADAV

SEQ ID NO: 10 - protein, 9 aa, synthetic construct
  REGION 1..9: note = neoantigen candidate (A0201) (Melanoma)
YIAGILARI

SEQ ID NO: 11 - protein, 11 aa, synthetic construct
  REGION 1..11: note = neoantigen candidate (A0201) (Melanoma)
RLAEFIIGMMG

SEQ ID NO: 12 - protein, 9 aa, synthetic construct
  REGION 1..9: note = neoantigen candidate (A0201) (Melanoma)
YLMVALASV

SEQ ID NO: 13 - protein, 12 aa, synthetic construct
  REGION 1..12: note = neoantigen candidate (A0201) (Melanoma)
RLAEFIIGMMGT

SEQ ID NO: 14 - protein, 9 aa, synthetic construct
  REGION 1..9: note = neoantigen candidate (A0201) (Melanoma)
GLVECLPEI

SEQ ID NO: 15 - protein, 10 aa, synthetic construct
  REGION 1..10: note = neoantigen candidate (A0201) (Melanoma)
AYLFNFVVNV

SEQ ID NO: 16 - protein, 9 aa, synthetic construct
  REGION 1..9: note = neoantigen candidate (A0201) (Melanoma)
VLFYLSSAV

SEQ ID NO: 17 - protein, 9 aa, synthetic construct
  REGION 1..9: note = neoantigen candidate (A0201) (Melanoma)
RLFFCFMNV

SEQ ID NO: 18 - protein, 9 aa, synthetic construct
  REGION 1..9: note = neoantigen candidate (A0201) (Melanoma)
CILAVLPSL

SEQ ID NO: 19 - protein, 9 aa, synthetic construct
  REGION 1..9: note = neoantigen candidate (A0201) (Melanoma)
IMFNKGFLA

SEQ ID NO: 20 - protein, 10 aa, synthetic construct
  REGION 1..10: note = neoantigen candidate (A0201) (Melanoma)
KTDPWFLLAV

SEQ ID NO: 21 - protein, 12 aa, synthetic construct
  REGION 1..12: note = neoantigen candidate (A0201) (Melanoma)
SLIGVSFFALPV

SEQ ID NO: 22 - protein, 10 aa, synthetic construct
  REGION 1..10: note = neoantigen candidate (A0201) (Melanoma)
SLWAESLVHV

SEQ ID NO: 23 - protein, 10 aa, synthetic construct
  REGION 1..10: note = neoantigen candidate (A0201) (Melanoma)
FLLAVLGAPV

SEQ ID NO: 24 - protein, 10 aa, synthetic construct
  REGION 1..10: note = neoantigen candidate (A2402) (Melanoma)
TFYWTFVNAF

SEQ ID NO: 25 - protein, 10 aa, synthetic construct
  REGION 1..10: note = neoantigen candidate (A2402) (Melanoma)
VFYQFSKLIF

SEQ ID NO: 26 - protein, 11 aa, synthetic construct
  REGION 1..11: note = neoantigen candidate (A2402) (Melanoma)
RMYSSWRLLNL

SEQ ID NO: 27 - protein, 10 aa, synthetic construct
  REGION 1..10: note = neoantigen candidate (A2402) (Melanoma)
TWNVHQQFLW

SEQ ID NO: 28 - protein, 9 aa, synthetic construct
  REGION 1..9: note = neoantigen candidate (A2402) (Melanoma)
RMYSSWRLL

SEQ ID NO: 29 - protein, 12 aa, synthetic construct
  REGION 1..12: note = neoantigen candidate (A2402) (Melanoma)
FYWTFVNAFSIF

SEQ ID NO: 30 - protein, 11 aa, synthetic construct
  REGION 1..11: note = neoantigen candidate (A2402) (Melanoma)
QWILKTRAYFL

SEQ ID NO: 31 - protein, 9 aa, synthetic construct
  REGION 1..9: note = neoantigen candidate (A2402) (Melanoma)
STWNVHQQF

SEQ ID NO: 32 - protein, 10 aa, synthetic construct
  REGION 1..10: note = neoantigen candidate (A2402) (Melanoma)
QWILKTRAYF

SEQ ID NO: 33 - protein, 11 aa, synthetic construct
  REGION 1..11: note = neoantigen candidate (A2402) (Melanoma)
STWNVHQQFLW

SEQ ID NO: 34 - protein, 9 aa, synthetic construct
  REGION 1..9: note = neoantigen candidate (A2402) (Melanoma)
FYWTFVNAF

SEQ ID NO: 35 - protein, 11 aa, synthetic construct
  REGION 1..11: note = neoantigen candidate (A2402) (Melanoma)
STWNVHQQFLW

SEQ ID NO: 36 - protein, 9 aa, synthetic construct
  REGION 1..9: note = neoantigen candidate (A2402) (Melanoma)
FYWTFVNAF

SEQ ID NO: 37 - protein, 11 aa, synthetic construct
  REGION 1..11: note = neoantigen candidate (A2402) (Melanoma)
STWNVHQQFLW

SEQ ID NO: 38 - protein, 9 aa, synthetic construct
  REGION 1..9: note = neoantigen candidate (A2402) (Melanoma)
FYWTFVNAF

SEQ ID NO: 39 - protein, 11 aa, synthetic construct
  REGION 1..11: note = neoantigen candidate (A2402) (Melanoma)
STWNVHQQFLW

SEQ ID NO: 40 - protein, 9 aa, synthetic construct
  REGION 1..9: note = neoantigen candidate (A2402) (Melanoma)
FYWTFVNAF

SEQ ID NO: 41 - protein, 11 aa, synthetic construct
  REGION 1..11: note = neoantigen candidate (A2402) (Melanoma)
STWNVHQQFLW

SEQ ID NO: 42 - protein, 9 aa, synthetic construct
  REGION 1..9: note = neoantigen candidate (A2402) (Melanoma)
FYWTFVNAF

SEQ ID NO: 43 - protein, 12 aa, synthetic construct
  REGION 1..12: note = neoantigen candidate (A2402) (Melanoma)
LYHFSDRMYSSW

SEQ ID NO: 44 - protein, 10 aa, synthetic construct
  REGION 1..10: note = neoantigen candidate (A1101) (Melanoma)
STACFHPVTK

SEQ ID NO: 45 - protein, 11 aa, synthetic construct
  REGION 1..11: note = neoantigen candidate (A1101) (Melanoma)
TTFGIQVRYLK

SEQ ID NO: 46 - protein, 11 aa, synthetic construct
  REGION 1..11: note = neoantigen candidate (A1101) (Melanoma)
KIGDFGLATMK

SEQ ID NO: 47 - protein, 11 aa, synthetic construct
  REGION 1..11: note = neoantigen candidate (A1101) (Melanoma)
KIGDFGLATEK

SEQ ID NO: 48 - protein, 10 aa, synthetic construct
  REGION 1..10: note = neoantigen candidate (A1101) (Melanoma)
SSSGSINLLK

SEQ ID NO: 49 - protein, 10 aa, synthetic construct
  REGION 1..10: note = neoantigen candidate (A1101) (Melanoma)
AVAVDFQFSK

SEQ ID NO: 50 - protein, 9 aa, synthetic construct
  REGION 1..9: note = neoantigen candidate (A1101) (Melanoma)
KTAPVEWRK

SEQ ID NO: 51 - protein, 10 aa, synthetic construct
  REGION 1..10: note = neoantigen candidate (A1101) (Melanoma)
STSYLQHREK

SEQ ID NO: 52 - protein, 9 aa, synthetic construct
  REGION 1..9: note = neoantigen candidate (A1101) (Melanoma)
VAVDFQFSK

SEQ ID NO: 53 - protein, 11 aa, synthetic construct
  REGION 1..11: note = neoantigen candidate (A1101) (Melanoma)
SAFTIQEYFVK

SEQ ID NO: 54 - protein, 10 aa, synthetic construct
  REGION 1..10: note = neoantigen candidate (A1101) (Melanoma)
SVSNTTVGSK

SEQ ID NO: 55 - protein, 9 aa, synthetic construct
  REGION 1..9: note = neoantigen candidate (A1101) (Melanoma)
RVQTGTIPK

SEQ ID NO: 56 - protein, 9 aa, synthetic construct
  REGION 1..9: note = neoantigen candidate (A1101) (Melanoma)
SSGSINLLK

SEQ ID NO: 57 - protein, 12 aa, synthetic construct
  REGION 1..12: note = neoantigen candidate (A1101) (Melanoma)
GTAAISVTGALK

SEQ ID NO: 58 - protein, 11 aa, synthetic construct
  REGION 1..11: note = neoantigen candidate (A1101) (Melanoma)
STPNFSRLRRY

SEQ ID NO: 59 - protein, 10 aa, synthetic construct
  REGION 1..10: note = neoantigen candidate (A1101) (Melanoma)
RSVLSSGYQK

SEQ ID NO: 60 - protein, 10 aa, synthetic construct
  REGION 1..10: note = neoantigen candidate (A1101) (Melanoma)
VVSPVSLPRR

SEQ ID NO: 61 - protein, 10 aa, synthetic construct
  REGION 1..10: note = neoantigen candidate (A1101) (Melanoma)
AAISVTGALK

SEQ ID NO: 62 - protein, 10 aa, synthetic construct
  REGION 1..10: note = neoantigen candidate (A1101) (Melanoma)
GSQPPSLGRK

SEQ ID NO: 63 - protein, 9 aa, synthetic construct
  REGION 1..9: note = neoantigen candidate (A1101) (Melanoma)
TVYCRYHNY

SEQ ID NO: 64 - protein, 10 aa, synthetic construct
  REGION 1..10: note = neoantigen candidate (MCF7-1)
LLFDMTTHSV

SEQ ID NO: 65 - protein, 9 aa, synthetic construct
  REGION 1..9: note = neoantigen candidate (MCF7-2)
FQSFFSLIV

SEQ ID NO: 66 - protein, 10 aa, synthetic construct
  REGION 1..10: note = neoantigen candidate (MCF7-3)
FLGSGVHGGV

SEQ ID NO: 67 - protein, 11 aa, synthetic construct
  REGION 1..11: note = neoantigen candidate (MCF7-4)
YLFFCGHMFHA

SEQ ID NO: 68 - protein, 9 aa, synthetic construct
  REGION 1..9: note = neoantigen candidate (MCF7-5)
ITFEHILAL

SEQ ID NO: 69 - protein, 9 aa, synthetic construct
  REGION 1..9: note = neoantigen candidate (MCF7-6)
NLANEITYI

SEQ ID NO: 70 - protein, 9 aa, synthetic construct
  REGION 1..9: note = neoantigen candidate (MCF7-7)
VLCEPVHGL

SEQ ID NO: 71 - protein, 10 aa, synthetic construct
  REGION 1..10: note = neoantigen candidate (MCF7-8)
MLLESLRHAV

SEQ ID NO: 72 - protein, 11 aa, synthetic construct
  REGION 1..11: note = neoantigen candidate (MCF7-9)
SLFGLGFEEHV

SEQ ID NO: 73 - protein, 10 aa, synthetic construct
  REGION 1..10: note = neoantigen candidate (MCF7-10)
HLLTDELGYV

SEQ ID NO: 74 - protein, 9 aa, synthetic construct
  REGION 1..9: note = neoantigen candidate (MCF7-11)
KLSEASMIV

SEQ ID NO: 75 - protein, 9 aa, synthetic construct
  REGION 1..9: note = neoantigen candidate (MCF7-12)
ALLDMRSLL

SEQ ID NO: 76 - protein, 11 aa, synthetic construct
  REGION 1..11: note = neoantigen candidate (MCF7-13)
GLWEALTPCNV

SEQ ID NO: 77 - protein, 9 aa, synthetic construct
  REGION 1..9: note = neoantigen candidate (MCF7-14)
SLARLHLTV

SEQ ID NO: 78 - protein, 9 aa, synthetic construct
  REGION 1..9: note = neoantigen candidate (MCF7-15)
TLLPLPLLL

SEQ ID NO: 79 - protein, 12 aa, synthetic construct
  REGION 1..12: note = neoantigen candidate (MCF7-16)
HLFWFADLNYRL

SEQ ID NO: 80 - protein, 11 aa, synthetic construct
  REGION 1..11: note = neoantigen candidate (MCF7-17)
STMSFLRSLYL

SEQ ID NO: 81 - protein, 9 aa, synthetic construct
  REGION 1..9: note = neoantigen candidate (MCF7-18)
TLNHEIYEA

SEQ ID NO: 82 - protein, 12 aa, synthetic construct
  REGION 1..12: note = neoantigen candidate (MCF7-19)
ILWGSISFNLAV

SEQ ID NO: 83 - protein, 9 aa, synthetic construct
  REGION 1..9: note = neoantigen candidate (MCF7-20)
MVCGAAFFI

SEQ ID NO: 84 - protein, 8 aa, synthetic construct
  REGION 1..8: note = neoantigen candidate (B16F10)
MSLPFSFL

SEQ ID NO: 85 - protein, 8 aa, synthetic construct
  REGION 1..8: note = neoantigen candidate (B16F10)
ANFIFRQL

SEQ ID NO: 86 - protein, 8 aa, synthetic construct
  REGION 1..8: note = neoantigen candidate (B16F10)
STYKLTNL

SEQ ID NO: 87 - protein, 8 aa, synthetic construct
  REGION 1..8: note = neoantigen candidate (B16F10)
NMYGFRNV

SEQ ID NO: 88 - protein, 8 aa, synthetic construct
  REGION 1..8: note = neoantigen candidate (B16F10)
VIYSHLQV

SEQ ID NO: 89 - protein, 8 aa, synthetic construct
  REGION 1..8: note = neoantigen candidate (B16F10)
SGFRYNVL

SEQ ID NO: 90 - protein, 8 aa, synthetic construct
  REGION 1..8: note = neoantigen candidate (B16F10)
VVMEYENL

SEQ ID NO: 91 - protein, 8 aa, synthetic construct
  REGION 1..8: note = neoantigen candidate (B16F10)
IVHYFIAL

SEQ ID NO: 92 - protein, 9 aa, synthetic construct
  REGION 1..9: note = neoantigen candidate (B16F10)
VSFAPLVQL

SEQ ID NO: 93 - protein, 9 aa, synthetic construct
  REGION 1..9: note = neoantigen candidate (B16F10)
ATFYFHHPV

SEQ ID NO: 94 - protein, 8 aa, synthetic construct
  REGION 1..8: note = neoantigen candidate (B16F10)
VHYLRLSL

SEQ ID NO: 95 - protein, 9 aa, synthetic construct
  REGION 1..9: note = neoantigen candidate (B16F10)
IGIFFQMRV

SEQ ID NO: 96 - protein, 8 aa, synthetic construct
  REGION 1..8: note = neoantigen candidate (B16F10)
VAHVAAFL

SEQ ID NO: 97 - protein, 8 aa, synthetic construct
  REGION 1..8: note = neoantigen candidate (B16F10)
VFLRVRAL

SEQ ID NO: 98 - protein, 8 aa, synthetic construct
  REGION 1..8: note = neoantigen candidate (B16F10)
TIFMMLRL

SEQ ID NO: 99 - protein, 8 aa, synthetic construct
  REGION 1..8: note = neoantigen candidate (B16F10)
KGFLYSAL

SEQ ID NO: 100 - protein, 8 aa, synthetic construct
  REGION 1..8: note = neoantigen candidate (B16F10)
SSVLFKGL

SEQ ID NO: 101 - protein, 8 aa, synthetic construct
  REGION 1..8: note = neoantigen candidate (B16F10)
MQFYLRHL

SEQ ID NO: 102 - protein, 8 aa, synthetic construct
  REGION 1..8: note = neoantigen candidate (B16F10)
ARMMFSGL

SEQ ID NO: 103 - protein, 9 aa, synthetic construct
  REGION 1..9: note = neoantigen candidate (B16F10)
KSLYYASCL

SEQ ID NO: 104 - protein, 8 aa, synthetic construct
  REGION 1..8: note = neoantigen candidate (B16F10)
LVFVVGRL

SEQ ID NO: 105 - protein, 8 aa, synthetic construct
  REGION 1..8: note = neoantigen candidate (B16F10)
SIGVYIPL

SEQ ID NO: 106 - protein, 8 aa, synthetic construct
  REGION 1..8: note = neoantigen candidate (B16F10)
TVYRCGHL

SEQ ID NO: 107 - protein, 9 aa, synthetic construct
  REGION 1..9: note = neoantigen candidate (B16F10)
SLFTLHQSV

SEQ ID NO: 108 - protein, 8 aa, synthetic construct
  REGION 1..8: note = neoantigen candidate (B16F10)
FTFVYPTI

SEQ ID NO: 109 - protein, 9 aa, synthetic construct
  REGION 1..9: note = neoantigen candidate (B16F10)
CMLRYQTCL

SEQ ID NO: 110 - protein, 9 aa, synthetic construct
  REGION 1..9: note = neoantigen candidate (B16F10)
VCFDYTFAL

SEQ ID NO: 111 - protein, 8 aa, synthetic construct
  REGION 1..8: note = neoantigen candidate (B16F10)
LNVYYLPL

SEQ ID NO: 112 - protein, 9 aa, synthetic construct
  REGION 1..9: note = neoantigen candidate (B16F10)
VPYAVFPPL

SEQ ID NO: 113 - protein, 8 aa, synthetic construct
  REGION 1..8: note = neoantigen candidate (B16F10)
VSFANAVV

SEQ ID NO: 114 - protein, 9 aa, synthetic construct
  REGION 1..9: note = neoantigen candidate (B16F10)
VVPSFSAEI

SEQ ID NO: 115 - protein, 10 aa, synthetic construct
  REGION 1..10: note = neoantigen candidate (B16F10)
CNFCYQRNQL

SEQ ID NO: 116 - protein, 9 aa, synthetic construct
  REGION 1..9: note = neoantigen candidate (B16F10)
QMYPAFKRV

SEQ ID NO: 117 - protein, 9 aa, synthetic construct
  REGION 1..9: note = neoantigen candidate (B16F10)
ILVSTYRPL

SEQ ID NO: 118 - protein, 9 aa, synthetic construct
  REGION 1..9: note = neoantigen candidate (B16F10)
SFLAGFRPL

SEQ ID NO: 119 - protein, 10 aa, synthetic construct
  REGION 1..10: note = neoantigen candidate (B16F10)
AIYHHASRAI

SEQ ID NO: 120 - protein, 10 aa, synthetic construct
  REGION 1..10: note = neoantigen candidate (B16F10)
IAMGFPVERL

SEQ ID NO: 121 - protein, 9 aa, synthetic construct
  REGION 1..9: note = neoantigen candidate (B16F10)
VLILHAAAL

SEQ ID NO: 122 - protein, 9 aa, synthetic construct
  REGION 1..9: note = neoantigen candidate (B16F10)
SLVAPFGSV

SEQ ID NO: 123 - protein, 8 aa, synthetic construct
  REGION 1..8: note = neoantigen candidate (B16F10)
MYRYFVTL

SEQ ID NO: 124 - protein, 9 aa, synthetic construct
  REGION 1..9: note = neoantigen candidate (B16F10)
VMMDNFDYL

SEQ ID NO: 125 - protein, 9 aa, synthetic construct
  REGION 1..9: note = neoantigen candidate (B16F10)
VTFQAFIDV

SEQ ID NO: 126 - protein, 8 aa, synthetic construct
  REGION 1..8: note = neoantigen candidate (B16F10)
RAFAAVRL

SEQ ID NO: 127 - protein, 12 aa, synthetic construct
  REGION 1..12: note = neoantigen candidate (B16F10)
KNFEFNKQRSIV

SEQ ID NO: 128 - protein, 12 aa, synthetic construct
  REGION 1..12: note = neoantigen candidate (B16F10)
LMYVYEMLGAGL

SEQ ID NO: 129 - protein, 10 aa, synthetic construct
  REGION 1..10: note = neoantigen candidate (B16F10)
CMLRYQTCLV

SEQ ID NO: 130 - protein, 8 aa, synthetic construct
  REGION 1..8: note = neoantigen candidate (B16F10)
AIALHLHL

SEQ ID NO: 131 - protein, 9 aa, synthetic construct
  REGION 1..9: note = neoantigen candidate (B16F10)
TSYSTAAPL

SEQ ID NO: 132 - protein, 10 aa, synthetic construct
  REGION 1..10: note = neoantigen candidate (B16F10)
SMPHYSSPAI

SEQ ID NO: 133 - protein, 9 aa, synthetic construct
  REGION 1..9: note = neoantigen candidate (B16F10)
TIPFYDNPI

SEQ ID NO: 134 - protein, 9 aa, synthetic construct
  REGION 1..9: note = mTRP2
SVYDFFVWL